European Patent Application EP 4 556 026 A1, published May 21, 2025. Title: 抗体药物偶联物及其制备方法和用途. Applicant: 苏州宜联生物医药有限公司. Application CN. The sequence listing filed with the application follows.

SEQUENCE LISTING (86 sequences)

SEQ ID NO: 1 - protein, 119 aa, synthetic construct
QIQLVQSGAELVRPGASVKMSCKTSGYTFTTYNVHWVKQTPRQGLEWIGAISPGNGLTSYTQKFKAKATLTVDKSSSTAYMQLSSLTSEDSAVYFCARGGFRLGSMDYWGQGTSVTVSS

SEQ ID NO: 2 - protein, 107 aa, synthetic construct
DIVMTQSHKFMSTSVGDRVSVTCKASQNVGTSVAWYQQRPGQSPKELIYWASNRFTGVPDRFTGSGSGTDFTLTITNVQSEDLADYFCQQYSSPPLTFGAGTKLELK

SEQ ID NO: 3 - protein, 5 aa, synthetic construct
TYNVH

SEQ ID NO: 4 - protein, 17 aa, synthetic construct
AISPGNGLTSYTQKFKA

SEQ ID NO: 5 - protein, 17 aa, synthetic construct
AISPGSGLTSYAQKFQG

SEQ ID NO: 6 - protein, 10 aa, synthetic construct
GGFRLGSMDY

SEQ ID NO: 7 - protein, 11 aa, synthetic construct
KASQNVGTSVA

SEQ ID NO: 8 - protein, 11 aa, synthetic construct
SASQNVGTSVA

SEQ ID NO: 9 - protein, 7 aa, synthetic construct
WASNRFT

SEQ ID NO: 10 - protein, 9 aa, synthetic construct
QQYSSPPLT

SEQ ID NO: 11 - protein, 8 aa, synthetic construct
GYTFTTYN

SEQ ID NO: 12 - protein, 8 aa, synthetic construct
ISPGNGLT

SEQ ID NO: 13 - protein, 8 aa, synthetic construct
ISPGSGLT

SEQ ID NO: 14 - protein, 12 aa, synthetic construct
ARGGFRLGSMDY

SEQ ID NO: 15 - protein, 6 aa, synthetic construct
QNVGTS

SEQ ID NO: 16 - protein, 9 aa, synthetic construct
QHYSKLPLT

SEQ ID NO: 17 - protein, 119 aa, synthetic construct
QVQLVESGAEVKQPGESVKVSCKTSGYTFTTYNVHWVRQAPGQGLEWMGAISPGSGLTSYAQKFQGRVTLTVDKSTSTAYMELSSLRSEDTAVYYCARGGFRLGSMDYWGQGTLVTVSS

SEQ ID NO: 18 - protein, 107 aa, synthetic construct
DIQMTQSPSFLSASVGDRVTITCSASQNVGTSVAWYQQKPGQSPKELIYWASNRFTGVPSRFSGSGSGTDFTLTISSLQPEDFATYYCQQYSSPPLTFGQGTKVEIK

SEQ ID NO: 19 - protein, 120 aa, synthetic construct
QAYLQQSGADLVRPGASVKMSSKASGSSFTTYIIHWIKQTPGQGLEWIGAIYPGNGYTSYNQKFKGKATLTVDKSYNTAYIQLSSLSSEDSAVYFCARGNYGNYEGFTYWGQGTLVTVSA

SEQ ID NO: 20 - protein, 107 aa, synthetic construct
DIQMTQTTSSLSVSLGDRITISCSASQAIYKYLNWYQQKPDGTVKLLIYYTSTLHSGVPSRFSGSGSGTDYSLTISNLEPEDIASYYCQQYNKFPFTFGSGTKLEIK

SEQ ID NO: 21 - protein, 5 aa, synthetic construct
TYIIH

SEQ ID NO: 22 - protein, 17 aa, synthetic construct
AIYPGNGYTSYNQKFKG

SEQ ID NO: 23 - protein, 17 aa, synthetic construct
AIYPGSGYTSYAQKFQG

SEQ ID NO: 24 - protein, 11 aa, synthetic construct
GNYGNYEGFTY

SEQ ID NO: 25 - protein, 11 aa, synthetic construct
SASQAIYKYLN

SEQ ID NO: 26 - protein, 7 aa, synthetic construct
YTSTLHS

SEQ ID NO: 27 - protein, 9 aa, synthetic construct
QQYNKFPFT

SEQ ID NO: 28 - protein, 8 aa, synthetic construct
GSSFTTYI

SEQ ID NO: 29 - protein, 8 aa, synthetic construct
IYPGNGYT

SEQ ID NO: 30 - protein, 8 aa, synthetic construct
IYPGSGYT

SEQ ID NO: 31 - protein, 13 aa, synthetic construct
ARGNYGNYEGFTY

SEQ ID NO: 32 - protein, 6 aa, synthetic construct
QAIYKY

SEQ ID NO: 33 - protein, 116 aa, synthetic construct
QVQLVESGPGLVQPSETLSLTCTVSGFSLTNYGVHWVRQPPGKGLEWIGVIWSGGRTNYNPSLQSRVTISKDNSTNQVSLKLSSVTAADTAVYYCAKRDGIYGDYWGQGTLVTVSS

SEQ ID NO: 34 - protein, 120 aa, synthetic construct
QVQLVESGAEVKQPGESVKVSCKASGSSFTTYIIHWIRQAPGQGLEWMGAIYPGSGYTSYAQKFQGRVTLTVDKSTSTAYMELSSLRSEDTAVYFCARGNYGNYEGFTYWGQGTLVTVSS

SEQ ID NO: 35 - protein, 107 aa, synthetic construct
DIQMTQSPSSLSASVGDRVTITCSASQAIYKYLNWYQQKPGQAPKLLIYYTSTLHSGVPSRFSGSGSGTDYTLTISSLQPEDFATYYCQQYNKFPFTFGQGTKVEIK

SEQ ID NO: 36 - protein, 119 aa, synthetic construct
QVQLQQSGAELVRPGASVKMSCKASGYTFTSNNLHWVKLTPRQGLEWIGAVYPGNGDTSYTQKFKGKATLTVDKSSSIAYMQLSSPTSEDSAVYFCARGLPYLGAMDYWGQGTSVTVSS

SEQ ID NO: 37 - protein, 107 aa, synthetic construct
DIVMTQSQRFMSTTVGDRVSITCKASQNVGIFVTWYQQKPGQSPKLLIYSASSRYTGVPDRFTGSGSGTDFTLTISNMQSEDLADYFCQQYSRSPLSFGAGTKLELK

SEQ ID NO: 38 - protein, 5 aa, synthetic construct
SNNLH

SEQ ID NO: 39 - protein, 17 aa, synthetic construct
AVYPGNGDTSYTQKFKG

SEQ ID NO: 40 - protein, 17 aa, synthetic construct
AVYPGSGDTSYSQKFQG

SEQ ID NO: 41 - protein, 10 aa, synthetic construct
GLPYLGAMDY

SEQ ID NO: 42 - protein, 11 aa, synthetic construct
KASQNVGIFVT

SEQ ID NO: 43 - protein, 11 aa, synthetic construct
SASQNVGIFVT

SEQ ID NO: 44 - protein, 7 aa, synthetic construct
SASSRYT

SEQ ID NO: 45 - protein, 9 aa, synthetic construct
QQYSRSPLS

SEQ ID NO: 46 - protein, 8 aa, synthetic construct
GYTFTSNN

SEQ ID NO: 47 - protein, 8 aa, synthetic construct
VYPGNGDT

SEQ ID NO: 48 - protein, 8 aa, synthetic construct
VYPGSGDT

SEQ ID NO: 49 - protein, 12 aa, synthetic construct
ARGLPYLGAMDY

SEQ ID NO: 50 - protein, 6 aa, synthetic construct
QNVGIF

SEQ ID NO: 51 - protein, 107 aa, synthetic construct
DIQMTQSPSSLSASVGDRVTITCSASQDIGTYLNWYQQKPGQAPKLLIYHTSRLHSGVPSRFSGSGSGTDFTLTISSLQPEDFATYYCQHYSKLPLTFGQGTKVEIK

SEQ ID NO: 52 - protein, 119 aa, synthetic construct
QVQLVESGAEVKQPGESVKVSCKASGYTFTSNNLHWVRQAPGQGLEWMGAVYPGSGDTSYSQKFQGRVTLTVDKSASTAYMELSSLRSEDTAVYFCARGLPYLGAMDYWGQGTLVTVSS

SEQ ID NO: 53 - protein, 107 aa, synthetic construct
DIQMTQSPSFLSASVGDRVTITCSASQNVGIFVTWYQQKPGQSPKLLIYSASSRYTGVPSRFSGSGSGTDFTLTISSLQPEDFATYYCQQYSRSPLSFGQGTKVEIK

SEQ ID NO: 54 - protein, 119 aa, synthetic construct
QVQLQQSGAELVRPGASVKMSCKASGYTFASYNMHWVKKTPRQGLEWIGAIYPGNGNTSYNQKFKGKATLTVDKSSSTAYMQLSSLTSEDSAVYFCVRGGRGLGTMDYWGQGTSVTVSS

SEQ ID NO: 55 - protein, 107 aa, synthetic construct
DIVMTQSHKFMSTSVGDRVSITCKASQDVGSSVAWYQQKPGQSPKLLIYWASTRHTGVPDRFTGSGSGTDFTLTISNVQSEDLADYFCQHYRNIPLTFGAGTKLELK

SEQ ID NO: 56 - protein, 5 aa, synthetic construct
SYNMH

SEQ ID NO: 57 - protein, 17 aa, synthetic construct
AIYPGNGNTSYNQKFKG

SEQ ID NO: 58 - protein, 17 aa, synthetic construct
AIYPGSGNTSYSQKFQG

SEQ ID NO: 59 - protein, 17 aa, synthetic construct
AIYPGSGNTGYSQKFQG

SEQ ID NO: 60 - protein, 10 aa, synthetic construct
GGRGLGTMDY

SEQ ID NO: 61 - protein, 11 aa, synthetic construct
KASQDVGSSVA

SEQ ID NO: 62 - protein, 11 aa, synthetic construct
SASQDVGSSVA

SEQ ID NO: 63 - protein, 7 aa, synthetic construct
WASTRHT

SEQ ID NO: 64 - protein, 9 aa, synthetic construct
QHYRNIPLT

SEQ ID NO: 65 - protein, 8 aa, synthetic construct
GYTFASYN

SEQ ID NO: 66 - protein, 8 aa, synthetic construct
IYPGNGNT

SEQ ID NO: 67 - protein, 8 aa, synthetic construct
IYPGSGNT

SEQ ID NO: 68 - protein, 12 aa, synthetic construct
VRGGRGLGTMDY

SEQ ID NO: 69 - protein, 6 aa, synthetic construct
QDVGSS

SEQ ID NO: 70 - protein, 330 aa, synthetic construct [sequence omitted]

SEQ ID NO: 71 - protein, 119 aa, synthetic construct
QVQLVESGAEVKQPGESVKVSCKASGYTFASYNMHWVRQAPGQGLEWMGAIYPGSGNTSYSQKFQGRVTLTVDKSASTAYMELSSLRSEDTAVYFCVRGGRGLGTMDYWGQGTLVTVSS

SEQ ID NO: 72 - protein, 107 aa, synthetic construct
DIQMTQSPSFLSASVGDRVTITCSASQDVGSSVAWYQQKPGQSPKLLIYWASTRHTGVPSRFSGSGSGTDFTLTISSLQPEDFATYYCQHYRNIPLTFGQGTKVEIK

SEQ ID NO: 73 - protein, 119 aa, synthetic construct
QVQLVESGAEVKQPGESVKVSCKASGYTFASYNMHWVRQAPGQGLEWMGAIYPGSGNTGYSQKFQGRVTLTVDKSASTAYMELSSLRSEDTAVYFCVRGGRGLGTMDYWGQGTLVTVSS

SEQ ID NO: 74 - protein, 116 aa, synthetic construct
QVQLKESGPVLVAPSQSLSITCTVSGFSLTNYGVHWVRQPPGKGLEWLGVIWSGGRTNYNSALMSRLSISKDNSKSQVFLKMNSLQTDDTAMYYCAKRDGIYGDYWGQGTSVTVSS

SEQ ID NO: 75 - protein, 107 aa, synthetic construct
DIQMTQTTSSLSASLGDRVTISCRASQDIGTYLNWYQQKPDGTVTLLIYHTSRLHSGVPSRFSGSGSGTDFSLTISSLEPEDIATYYCQHYSKLPLTFGAGTKLELK

SEQ ID NO: 76 - protein, 8 aa, synthetic construct
GFSLTNYG

SEQ ID NO: 77 - protein, 7 aa, synthetic construct
IWSGGRT

SEQ ID NO: 78 - protein, 10 aa, synthetic construct
AKRDGIYGDY

SEQ ID NO: 79 - protein, 6 aa, synthetic construct
QDIGTY

SEQ ID NO: 80 - protein, 107 aa, synthetic construct [sequence omitted]

SEQ ID NO: 81 - protein, 449 aa, synthetic construct
QVQLVESGAEVKQPGESVKVSCKASGYTFASYNMHWVRQAPGQGLEWMGAIYPGSGNTGYSQKFQGRVTLTVDKSASTAYMELSSLRSEDTAVYFCVRGGRGLGTMDYWGQGTLVTVSSASTKGPSVFPLAPSSKSTSGGTAALGCLVKDYFPEPVTVSWNSGALTSGVHTFPAVLQSSGLYSLSSVVTVPSSSLGTQTYICNVNHKPSNTKVDKKVEPKSCDKTHTCPPCPAPELLGGPSVFLFPPKPKDTLMISRTPEVTCVVVDVSHEDPEVKFNWYVDGVEVHNAKTKPREEQYNSTYRVVSVLTVLHQDWLNGKEYKCKVSNKALPAPIEKTISKAKGQPREPQVYTLPPSRDELTKNQVSLTCLVKGFYPSDIAVEWESNGQPENNYKTTPPVLDSDGSFFLYSKLTVDKSRWQQGNVFSCSVMHEALHNHYTQKSLSLSPGK

SEQ ID NO: 82 - protein, 214 aa, synthetic construct
DIQMTQSPSFLSASVGDRVTITCSASQDVGSSVAWYQQKPGQSPKLLIYWASTRHTGVPSRFSGSGSGTDFTLTISSLQPEDFATYYCQHYRNIPLTFGQGTKVEIKRTVAAPSVFIFPPSDEQLKSGTASVVCLLNNFYPREAKVQWKVDNALQSGNSQESVTEQDSKDSTYSLSSTLTLSKADYEKHKVYACEVTHQGLSSPVTKSFNRGEC

SEQ ID NO: 83 - protein, 449 aa, synthetic construct
QVQLVESGAEVKQPGESVKVSCKTSGYTFTTYNVHWVRQAPGQGLEWMGAISPGSGLTSYAQKFQGRVTLTVDKSTSTAYMELSSLRSEDTAVYYCARGGFRLGSMDYWGQGTLVTVSSASTKGPSVFPLAPSSKSTSGGTAALGCLVKDYFPEPVTVSWNSGALTSGVHTFPAVLQSSGLYSLSSVVTVPSSSLGTQTYICNVNHKPSNTKVDKKVEPKSCDKTHTCPPCPAPELLGGPSVFLFPPKPKDTLMISRTPEVTCVVVDVSHEDPEVKFNWYVDGVEVHNAKTKPREEQYNSTYRVVSVLTVLHQDWLNGKEYKCKVSNKALPAPIEKTISKAKGQPREPQVYTLPPSRDELTKNQVSLTCLVKGFYPSDIAVEWESNGQPENNYKTTPPVLDSDGSFFLYSKLTVDKSRWQQGNVFSCSVMHEALHNHYTQKSLSLSPGK

SEQ ID NO: 84 - protein, 214 aa, synthetic construct
DIQMTQSPSFLSASVGDRVTITCSASQNVGTSVAWYQQKPGQSPKELIYWASNRFTGVPSRFSGSGSGTDFTLTISSLQPEDFATYYCQQYSSPPLTFGQGTKVEIKRTVAAPSVFIFPPSDEQLKSGTASVVCLLNNFYPREAKVQWKVDNALQSGNSQESVTEQDSKDSTYSLSSTLTLSKADYEKHKVYACEVTHQGLSSPVTKSFNRGEC

SEQ ID NO: 85 - protein, 231 aa, synthetic construct
PKSSDKTHTCPPCPAPELLGGPSVFLFPPKPKDTLMISRTPEVTCVVVDVSHEDPEVKFNWYVDGVEVHNAKTKPREEQYNSTYRVVSVLTVLHQDWLNGKEYKCKVSNKALPAPIEKTISKAKGQPREPQVYTLPPSRDELTKNQVSLTCLVKGFYPSDIAVEWESNGQPENNYKTTPPVLDSDGSFFLYSKLTVDKSRWQQGNVFSCSVMHEALHNHYTQKSLSLSPGK

SEQ ID NO: 86 - protein, 237 aa, synthetic construct
GGGGSPRGPTIKPCPPCKCPAPNLLGGPSVFIFPPKIKDVLMISLSPIVTCVVVDVSEDDPDVQISWFVNNVEVHTAQTQTHREDYNSTLRVVSALPIQHQDWMSGKEFKCKVNNKDLPAPIERTISKPKGSVRAPQVYVLPPPEEEMTKKQVTLTCMVTDFMPEDIYVEWTNNGKTELNYKNTEPVLDSDGSYFMYSKLRVEKKNWVERNSYSCSVVHEGLHNHHTTKSFSRTPGK